European Patent Application EP 4 733 413 A1, published April 29, 2026. Title: BIOMARKERS FOR HYPOXIC-ISCHEMIC ENCEPHALOPATHY, AND DIAGNOSTIC METHODS USING THEREOF. Applicant: COMMISSARIAT A L ENERGIE ATOMIQUE ET AUX ENERGIES ALTERNATIVES. Application EP. The sequence listing filed with the application follows.

SEQUENCE LISTING (30 sequences)

SEQ ID NO: 1 - DNA, 22 bp, synthetic construct
  source 1..22: mol_type = other DNA; note = GFAP forward qPCR primer
gctaatgactatcgccgccaac

SEQ ID NO: 2 - DNA, 22 bp, synthetic construct
  source 1..22: mol_type = other DNA; note = GFAP reverse qPCR primer
gcatttgcctctccaaggactc

SEQ ID NO: 3 - DNA, 22 bp, synthetic construct
  source 1..22: mol_type = other DNA; note = IBA1 forward qPCR primer
atcgtcatctccccacctaagg

SEQ ID NO: 4 - DNA, 22 bp, synthetic construct
  source 1..22: mol_type = other DNA; note = IBA1 reverse qPCR primer
tcccatccaacctctcttcctg

SEQ ID NO: 5 - DNA, 21 bp, synthetic construct
  source 1..21: mol_type = other DNA; note = MAP2 forward qPCR primer
cggaaaaccacagcaacaagt

SEQ ID NO: 6 - DNA, 20 bp, synthetic construct
  source 1..20: mol_type = other DNA; note = MAP2 reverse qPCR primer
ggtcttgggagggaagaacg

SEQ ID NO: 7 - DNA, 20 bp, synthetic construct
  source 1..20: mol_type = other DNA; note = NEUN forward qPCR primer
agcacagacagatagccagc

SEQ ID NO: 8 - DNA, 20 bp, synthetic construct
  source 1..20: mol_type = other DNA; note = NEUN reverse qPCR primer
tttcccgaattgcccgaaca

SEQ ID NO: 9 - DNA, 19 bp, synthetic construct
  source 1..19: mol_type = other DNA; note = VEGFA forward qPCR primer
ccacttctgaggagcctag

SEQ ID NO: 10 - DNA, 18 bp, synthetic construct
  source 1..18: mol_type = other DNA; note = VEGFA reverse qPCR primer
ggaggaggagccattacc

SEQ ID NO: 11 - DNA, 20 bp, synthetic construct
  source 1..20: mol_type = other DNA; note = ANGT1 forward qPCR primer
tgctaacaggaggttggtgg

SEQ ID NO: 12 - DNA, 20 bp, synthetic construct
  source 1..20: mol_type = other DNA; note = ANGT1 reverse qPCR primer
ttttccatggttttgccccg

SEQ ID NO: 13 - DNA, 20 bp, synthetic construct
  source 1..20: mol_type = other DNA; note = ANGT2 forward qPCR primer
gacggctgtgatgatcgaga

SEQ ID NO: 14 - DNA, 22 bp, synthetic construct
  source 1..22: mol_type = other DNA; note = ANGT2 reverse qPCR primer
cgtctggtttagtacttgggct

SEQ ID NO: 15 - DNA, 21 bp, synthetic construct
  source 1..21: mol_type = other DNA; note = APCDD1 forward qPCR primer
ctgcagaacgccaagaatcac

SEQ ID NO: 16 - DNA, 20 bp, synthetic construct
  source 1..20: mol_type = other DNA; note = APCDD1 reverse qPCR primer
cattccccatggaggccaat

SEQ ID NO: 17 - DNA, 20 bp, synthetic construct
  source 1..20: mol_type = other DNA; note = PACS1 forward qPCR primer
cctgcaggcataagttccct

SEQ ID NO: 18 - DNA, 20 bp, synthetic construct
  source 1..20: mol_type = other DNA; note = PACS1 reverse qPCR primer
ggagggcgagtcttcaacaa

SEQ ID NO: 19 - DNA, 20 bp, synthetic construct
  source 1..20: mol_type = other DNA; note = LETM1 forward qPCR primer
ggttgacgagccatgagagt

SEQ ID NO: 20 - DNA, 20 bp, synthetic construct
  source 1..20: mol_type = other DNA; note = LETM1 reverse qPCR primer
caggcctctgagtccaacag

SEQ ID NO: 21 - DNA, 21 bp, synthetic construct
  source 1..21: mol_type = other DNA; note = VWF forward qPCR primer
ccagccacattccatacaatc

SEQ ID NO: 22 - DNA, 23 bp, synthetic construct
  source 1..23: mol_type = other DNA; note = VWF reverse qPCR primer
ccaatcaacacagactccattag

SEQ ID NO: 23 - DNA, 20 bp, synthetic construct
  source 1..20: mol_type = other DNA; note = AGRIN forward qPCR primer
tgccgtaagggatgactgtg

SEQ ID NO: 24 - DNA, 20 bp, synthetic construct
  source 1..20: mol_type = other DNA; note = AGRIN reverse qPCR primer
caggtgtcatgggatctgct

SEQ ID NO: 25 - DNA, 20 bp, synthetic construct
  source 1..20: mol_type = other DNA; note = SLC17A7 forward qPCR primer
acagccttttgcggttccta

SEQ ID NO: 26 - DNA, 20 bp, synthetic construct
  source 1..20: mol_type = other DNA; note = SLC17A7 reverse qPCR primer
cccgaagctgccatagacat

SEQ ID NO: 27 - DNA, 20 bp, synthetic construct
  source 1..20: mol_type = other DNA; note = GABBR1 forward qPCR primer
ctacaatgtcgcggtcctgt

SEQ ID NO: 28 - DNA, 20 bp, synthetic construct
  source 1..20: mol_type = other DNA; note = GABBR1 reverse qPCR primer
ggcacaaagagcacaaccag

SEQ ID NO: 29 - DNA, 20 bp, synthetic construct
  source 1..20: mol_type = other DNA; note = TXN2 forward qPCR primer
atttgcctctggtgtatttc

SEQ ID NO: 30 - DNA, 23 bp, synthetic construct
  source 1..23: mol_type = other DNA; note = TXN2 reverse qPCR primer
ttatccattactctcacttgttc